European Patent Specification EP 4 034 674 B1, published March 26, 2025. Title: Probe and method for STR-genotyping. Applicant: Universiteit Gent. The sequence listing filed with the application follows.

SEQUENCE LISTING (26 sequences)

SEQ ID NO: 1 - DNA, 24 bp, Primer
gggggtctaagagcttgtaaaaag

SEQ ID NO: 2 - DNA, 29 bp, Primer
gtttgtgtgtgcatctgtaagcatgtatc

SEQ ID NO: 3 - DNA, 56 bp, Probe
gttttgtctttcaatgatatctatctatctatctatctatctatctatctatccac

SEQ ID NO: 4 - DNA, 60 bp, Probe
gttttgtctttcaatgatatctatctatctatctatctatctatctatctatctatccac

SEQ ID NO: 5 - DNA, 64 bp, Probe
gttttgtctttcaatgatatctatctatctatctatctatctatctatctatctatctatccac

SEQ ID NO: 6 - DNA, 68 bp, Probe
gttttgtctttcaatgatatctatctatctatctatctatctatctatctatctatctatctatccac

SEQ ID NO: 7 - DNA, 72 bp, Probe
gttttgtctttcaatgatatctatctatctatctatctatctatctatctatctatctatctatctatccac

SEQ ID NO: 8 - DNA, 21 bp, Primer
gtgattcccattggcctgttc

SEQ ID NO: 9 - DNA, 29 bp, Primer
gtttgtgtgtgcatctgtaagcatgtatc

SEQ ID NO: 10 - DNA, 52 bp, Probe
cctcattcattcattcattcattcattcaccatggagtctgtgttccctgtg

SEQ ID NO: 11 - DNA, 56 bp, Probe
cctcattcattcattcattcattcattcattcaccatggagtctgtgttccctgtg

SEQ ID NO: 12 - DNA, 60 bp, Probe
cctcattcattcattcattcattcattcattcattcaccatggagtctgtgttccctgtg

SEQ ID NO: 13 - DNA, 64 bp, Probe
cctcattcattcattcattcattcattcattcattcattcaccatggagtctgtgttccctgtg

SEQ ID NO: 14 - DNA, 68 bp, Probe
cctcattcattcattcattcattcattcattcattcattcattcaccatggagtctgtgttccctgtg

SEQ ID NO: 15 - DNA, 67 bp, Probe 9.3
cctcattcattcattcatcattcattcattcattcattcattcaccatggagtctgtgttccctgtg

SEQ ID NO: 16 - DNA, 32 bp, Forward primer
attgcaacttatatgtatttttgtatttcatg

SEQ ID NO: 17 - DNA, 28 bp, Reverse primer
accaaattgtgttcatgagtatagtttc

SEQ ID NO: 18 - DNA, 69 bp, Probe 10
ttgtatttcatgtgtacattcgtatctatctatctatctatctatctatctatctatctatctattccc

SEQ ID NO: 19 - DNA, 73 bp, Probe 11
ttgtatttcatgtgtacattcgtatctatctatctatctatctatctatctatctatctatctatctattccc

SEQ ID NO: 20 - DNA, 77 bp, Probe 12
ttgtatttcatgtgtacattcgtatctatctatctatctatctatctatctatctatctatctatctatctattccc

SEQ ID NO: 21 - DNA, 81 bp, Probe 13
ttgtatttcatgtgtacattcgtatctatctgtctatctatctatctatctatctatctatctatctatctatctattccc

SEQ ID NO: 22 - DNA, 81 bp, Probe 13'
ttgtatttcatgtgtacattcgtatctatctatctatctatctatctatctatctatctatctatctatctatctattccc

SEQ ID NO: 23 - DNA, 85 bp, Probe 14
ttgtatttcatgtgtacattcgtatctatctgtctatctatctatctatctatctatctatctatctatctatctatctattccc

SEQ ID NO: 24 - DNA, 85 bp, Probe 14'
ttgtatttcatgtgtacattcgtatctatctatctatctatctatctatctatctatctatctatctatctatctatctattccc

SEQ ID NO: 25 - DNA, 89 bp, Probe 15
ttgtatttcatgtgtacattcgtatctatctgtctatctatctatctatctatctatctatctatctatctatctatctatctattccc

SEQ ID NO: 26 - DNA, 93 bp, Probe 16
ttgtatttcatgtgtacattcgtatctatctgtctatctatctatctatctatctatctatctatctatctatctatctatctatctattccc